European Patent Application EP 4 368 712 A1, published May 15, 2024. Title: PREPARATION METHOD FOR AND APPLICATION OF IMMOBILIZED CELLS FOR MANNOSE PRODUCTION. Applicant: TIANJIN INSTITUTE OF INDUSTRIAL BIOTECHNOLOGY, CHINESE ACADEMY OF SCIENCES. The sequence listing filed with the application follows.

SEQUENCE LISTING (20 sequences)

SEQ ID NO: 1 - DNA, 50 bp, Artificial Sequence
  primer
agaaacaacaaagggggagatttgtatggtgaacgtttccaatgccgttg

SEQ ID NO: 2 - DNA, 51 bp, Artificial Sequence
  primer
gcttgagctcgactctagaggatcctcagtcaagtcccttccacttgacca

SEQ ID NO: 3 - DNA, 51 bp, Artificial Sequence
  primer
tggtcaagtggaagggacttgactgaggatcctctagagtcgagctcaagc

SEQ ID NO: 4 - DNA, 50 bp, Artificial Sequence
  primer
caacggcattggaaacgttcaccatacaaatctccccctttgttgtttct

SEQ ID NO: 5 - DNA, 50 bp, Artificial Sequence
  primer
agaaacaacaaagggggagatttgtatgggcaaactgtttggtaccttcg

SEQ ID NO: 6 - DNA, 50 bp, Artificial Sequence
  primer
gcttgagctcgactctagaggatccttaacctttcagtgcttcttccagc

SEQ ID NO: 7 - DNA, 51 bp, Artificial Sequence
  primer
gctggaagaagcactgaaaggttaaggatcctctagagtcgagctcaagct

SEQ ID NO: 8 - DNA, 50 bp, Artificial Sequence
  primer
cgaaggtaccaaacagtttgcccatacaaatctccccctttgttgtttct

SEQ ID NO: 9 - DNA, 50 bp, Artificial Sequence
  primer
agaaacaacaaagggggagatttgtatgctgcgtctggatactcgctttc

SEQ ID NO: 10 - DNA, 51 bp, Artificial Sequence
  primer
agcttgagctcgactctagaggatccttaaccagccaggcgtttacgagtc

SEQ ID NO: 11 - DNA, 51 bp, Artificial Sequence
  primer
gactcgtaaacgcctggctggttaaggatcctctagagtcgagctcaagct

SEQ ID NO: 12 - DNA, 50 bp, Artificial Sequence
  primer
gaaagcgagtatccagacgcagcatacaaatctccccctttgttgtttct

SEQ ID NO: 13 - DNA, 56 bp, Artificial Sequence
  primer
gtagaaacaacaaagggggagatttgtatgaggcggttggagcccaaacccgtggc

SEQ ID NO: 14 - DNA, 55 bp, Artificial Sequence
  primer
ccacgggtttgggctccaaccgcctcatacaaatctccccctttgttgtttctac

SEQ ID NO: 15 - DNA, 53 bp, Artificial Sequence
  primer
tgccgccctggccaaggagggggcgtgaggatcctctagagtcgagctcaagc

SEQ ID NO: 16 - DNA, 53 bp, Artificial Sequence
  primer
gcttgagctcgactctagaggatcctcacgccccctccttggccagggcggca

SEQ ID NO: 17 - DNA, 52 bp, Artificial Sequence
  primer
gtagaaacaacaaagggggagatttgtatgtaccgcgtttttgtttttgatc

SEQ ID NO: 18 - DNA, 52 bp, Artificial Sequence
  primer
gatcaaaaacaaaaacgcggtacatacaaatctccccctttgttgtttctac

SEQ ID NO: 19 - DNA, 49 bp, Artificial Sequence
  primer
agcaccgattgtctggatgaatgaggatcctctagagtcgagctcaagc

SEQ ID NO: 20 - DNA, 49 bp, Artificial Sequence
  primer
gcttgagctcgactctagaggatcctcattcatccagacaatcggtgct